European Patent Specification EP 3 507 373 B1, published September 13, 2023. Title: GENETICALLY MODIFIED NON-HUMAN ANIMAL WITH  HUMAN OR CHIMERIC PD-L1. Applicant: Beijing Biocytogen Co., Ltd. The sequence listing filed with the application follows.

SEQUENCE LISTING (68 sequences)

SEQ ID NO: 1 - DNA, 23 bp, Artificial Sequence
gtatggcagcaacgtcacgatgg

SEQ ID NO: 2 - DNA, 23 bp, Artificial Sequence
gcttgcgttagtggtgtactggg

SEQ ID NO: 3 - DNA, 23 bp, Artificial Sequence
gctggacctgcttgcgttagtgg

SEQ ID NO: 4 - DNA, 23 bp, Artificial Sequence
aggtccagctcccgttctacagg

SEQ ID NO: 5 - DNA, 23 bp, Artificial Sequence
gtttactatcacggctccaaagg

SEQ ID NO: 6 - DNA, 23 bp, Artificial Sequence
ggctccaaaggacttgtacgtgg

SEQ ID NO: 7 - DNA, 23 bp, Artificial Sequence
cgtgatagtaaacgctgaaaagg

SEQ ID NO: 8 - DNA, 23 bp, Artificial Sequence
attccctgtagaacgggagctgg

SEQ ID NO: 9 - DNA, 23 bp, Artificial Sequence
gacttgtacgtggtggagtatgg

SEQ ID NO: 10 - DNA, 23 bp, Artificial Sequence
tgctgcataatcagctacggtgg

SEQ ID NO: 11 - DNA, 23 bp, Artificial Sequence
cataatcagctacggtggtgcgg

SEQ ID NO: 12 - DNA, 23 bp, Artificial Sequence
gacgtcaagctgcaggacgcagg

SEQ ID NO: 13 - DNA, 23 bp, Artificial Sequence
tactgctgcataatcagctacgg

SEQ ID NO: 14 - DNA, 23 bp, Artificial Sequence
gatcacagacgtcaagctgcagg

SEQ ID NO: 15 - DNA, 23 bp, Artificial Sequence
gcttgacgtctgtgatctgaagg

SEQ ID NO: 16 - DNA, 23 bp, Artificial Sequence
cagcatttcccttcaaaagctgg

SEQ ID NO: 17 - DNA, 19 bp, Artificial Sequence
tatggcagcaacgtcacga

SEQ ID NO: 18 - DNA, 27 bp, Artificial Sequence
taggtaggtatggcagcaacgtcacga

SEQ ID NO: 19 - DNA, 19 bp, Artificial Sequence
tcgtgacgttgctgccata

SEQ ID NO: 20 - DNA, 23 bp, Artificial Sequence
aaactcgtgacgttgctgccata

SEQ ID NO: 21 - DNA, 18 bp, Artificial Sequence
ctgcataatcagctacgg

SEQ ID NO: 22 - DNA, 22 bp, Artificial Sequence
taggctgcataatcagctacgg

SEQ ID NO: 23 - DNA, 18 bp, Artificial Sequence
ccgtagctgattatgcag

SEQ ID NO: 24 - DNA, 22 bp, Artificial Sequence
aaacccgtagctgattatgcag

SEQ ID NO: 25 - DNA, 132 bp, Artificial Sequence
gaattctaatacgactcactatagggggtcttcgagaagacctgttttagagctagaaatagcaagttaaaataaggctagtccgttatcaacttgaaaaagtggcaccgagtcggtgcttttaaaggatcc

SEQ ID NO: 26 - DNA, 3653 bp, Mouse
gaaatcgtggtccccaagcctcatgccaggctgcacttgcacgtcgcgggccagtctcctcgcctgcagatagttcccaaaacatgaggatatttgctggcattatattcacagcctgctgtcacttgctacgggcgtttactatcacggctccaaaggacttgtacgtggtggagtatggcagcaacgtcacgatggagtgcagattccctgtagaacgggagctggacctgcttgcgttagtggtgtactgggaaaaggaagatgagcaagtgattcagtttgtggcaggagaggaggaccttaagcctcagcacagcaacttcagggggagagcctcgctgccaaaggaccagcttttgaagggaaatgctgcccttcagatcacagacgtcaagctgcaggacgcaggcgtttactgctgcataatcagctacggtggtgcggactacaagcgaatcacgctgaaagtcaatgccccataccgcaaaatcaaccagagaatttccgtggatccagccacttctgagcatgaactaatatgtcaggccgagggttatccagaagctgaggtaatctggacaaacagtgaccaccaacccgtgagtgggaagagaagtgtcaccacttcccggacagaggggatgcttctcaatgtgaccagcagtctgagggtcaacgccacagcgaatgatgttttctactgtacgttttggagatcacagccagggcaaaaccacacagcggagctgatcatcccagaactgcctgcaacacatcctccacagaacaggactcactgggtgcttctgggatccatcctgttgttcctcattgtagtgtccacggtcctcctcttcttgagaaaacaagtgagaatgctagatgtggagaaatgtggcgttgaagatacaagctcaaaaaaccgaaatgatacacaattcgaggagacgtaagcagtgttgaaccctctgatcgtcgattggcagcttgtggtctgtgaaagaaagggcccatgggacatgagtccaaagactcaagatggaacctgagggagagaaccaagaaagtgttgggagaggagcctggaacaacggacattttttccagggagacactgctaagcaagttgcccatcagtcgtcttgggaaatggattgagggttcctggcttagcagctggtccttgcacagtgaccttttcctctgctcagtgccgggatgagagatggagtcatgagtgttgaagaataagtgccttctatttattttgagtctgtgtgttctcactttgggcatgtaattatgactggtgaattctgacgacatgatagatcttaagatgtagtcaccaaactcaactgctgcttagcatcctccgtaactactgatacaagcagggaacacagaggtcacctgcttggtttgacaggctcttgctgtctgactcaaataatctttatttttcagtcctcaaggctcttcgatagcagttgttctgtatcagccttataggtgtcaggtatagcactcaacatctcatctcattacaatagcaaccctcatcaccatagcaacagctaacctctgttatcctcacttcatagccaggaagctgagcgactaagtcacttgcccacagagtatcagctctcagatttctgttcttcagccactgtcctttcaggatagaatttgtcgttaagaaattaatttaaaaactgattattgagtagcattgtatatcaatcacaacatgccttgtgcactgtgctggcctctgagcataaagatgtacgccggagtaccggtcggacatgtttatgtgtgttaaatactcagagaaatgttcattaacaaggagcttgcattttagagacactggaaagtaactccagttcattgtctagcattacatttacctcatttgctatccttgccatacagtctcttgttctccatgaagtgtcatgaatcttgttgaatagttcttttattttttaaatgtttctatttaaatgatattgacatctgaggcgatagctcagttggtaaaaccctttcctcacaagtgtgaaaccctgagtcttatccctagaacccacataaaaaacagttgcgtatgtttgtgcatgcttttgatcccagcactagggaggcagaggcaggcagatcctgagctctcattgaccacccagcctagcctacatggttagctccaggcctacaggagctggcagagcctgaaaaacgatgcctagacacacacacacacacacacacacacacacacacacacacacaccatgtactcatagacctaagtgcaccctcctacacatgcacacacatacaattcaaacacaaatcaacagggaattgtctcagaatggtccccaagacaaagaagaagaaaaacaccaaaccagctctattccctcagcctatcctctctactccttcctagaagcaactactattgtttttgtatataaatttacccaacgacagttaatatgtagaatatatattaaagtgtctgtcaatatatattatctctttctttctttcttcctttctttctttctttctttctttctttctttctttctttctttctttcttccttccttccttccttccttccttccttccttcctttctttctttctttctttttttctgtctatctgtacctaaatggttgctcactatgcattttctgtgctcttcgccctttttatttaatgtatggatatttatgctgcttccagaatggatctaaagctctttgtttctaggttttctcccccatccttctaggcatctctcacactgtctaggccagacaccatgtctgctgcctgaatctgtagacaccatttataaagcacgtactcaccgagtttgtatttggcttgttctgtgtctgattaaagggagaccatgagtccccagggtacactgagttaccccagtaccaagggggagccttgtttgtgtctccatggcagaagcaggcctggagccattttggtttcttccttgacttctctcaaacacagacgcctcacttgctcattacaggttctcctttgggaatgtcagcattgctccttgactgctggctgccctggaaggagcccattagctctgtgtgagcccttgacagctactgcctctccttaccacaggggcctctaagatactgttacctagaggtcttgaggatctgtgttctctggggggaggaaaggaggaggaacccagaactttcttacagttttccttgttctgtcacatgtcaagactgaaggaacaggctgggctacgtagtgagatcctgtctcaaaggaaagacgagcatagccgaacccccggtggaaccccctctgttacctgttcacacaagcttattgatgagtctcatgttaatgtcttgtttgtatgaagtttaagaaaatatcgggttgggcaacacattctatttattcattttatttgaaatcttaatgccatctcatggtgttggattggtgtggcactttattcttttgtgttgtgtataaccataaattttattttgcatcagattgtcaatgtattgcattaatttaataaatatttttatttattaaaaaaaaaaaaaaaaa

SEQ ID NO: 27 - protein, 290 aa, Mouse
MRIFAGIIFTACCHLLRAFTITAPKDLYVVEYGSNVTMECRFPVERELDLLALVVYWEKEDEQVIQFVAGEEDLKPQHSNFRGRASLPKDQLLKGNAALQITDVKLQDAGVYCCIISYGGADYKRITLKVNAPYRKINQRISVDPATSEHELICQAEGYPEAEVIWTNSDHQPVSGKRSVTTSRTEGMLLNVTSSLRVNATANDVFYCTFWRSQPGQNHTAELIIPELPATHPPQNRTHWVLLGSILLFLIVVSTVLLFLRKQVRMLDVEKCGVEDTSSKNRNDTQFEET

SEQ ID NO: 28 - DNA, 3691 bp, human
ggcgcaacgctgagcagctggcgcgtcccgcgcggccccagttctgcgcagcttcccgaggctccgcaccagccgcgcttctgtccgcctgcagggcattccagaaagatgaggatatttgctgtctttatattcatgacctactggcatttgctgaacgcatttactgtcacggttcccaaggacctatatgtggtagagtatggtagcaatatgacaattgaatgcaaattcccagtagaaaaacaattagacctggctgcactaattgtctattgggaaatggaggataagaacattattcaatttgtgcatggagaggaagacctgaaggttcagcatagtagctacagacagagggcccggctgttgaaggaccagctctccctgggaaatgctgcacttcagatcacagatgtgaaattgcaggatgcaggggtgtaccgctgcatgatcagctatggtggtgccgactacaagcgaattactgtgaaagtcaatgccccatacaacaaaatcaaccaaagaattttggttgtggatccagtcacctctgaacatgaactgacatgtcaggctgagggctaccccaaggccgaagtcatctggacaagcagtgaccatcaagtcctgagtggtaagaccaccaccaccaattccaagagagaggagaagcttttcaatgtgaccagcacactgagaatcaacacaacaactaatgagattttctactgcacttttaggagattagatcctgaggaaaaccatacagctgaattggtcatcccagaactacctctggcacatcctccaaatgaaaggactcacttggtaattctgggagccatcttattatgccttggtgtagcactgacattcatcttccgtttaagaaaagggagaatgatggatgtgaaaaaatgtggcatccaagatacaaactcaaagaagcaaagtgatacacatttggaggagacgtaatccagcattggaacttctgatcttcaagcagggattctcaacctgtggtttaggggttcatcggggctgagcgtgacaagaggaaggaatgggcccgtgggatgcaggcaatgtgggacttaaaaggcccaagcactgaaaatggaacctggcgaaagcagaggaggagaatgaagaaagatggagtcaaacagggagcctggagggagaccttgatactttcaaatgcctgaggggctcatcgacgcctgtgacagggagaaaggatacttctgaacaaggagcctccaagcaaatcatccattgctcatcctaggaagacgggttgagaatccctaatttgagggtcagttcctgcagaagtgccctttgcctccactcaatgcctcaatttgttttctgcatgactgagagtctcagtgttggaacgggacagtatttatgtatgagtttttcctatttattttgagtctgtgaggtcttcttgtcatgtgagtgtggttgtgaatgatttcttttgaagatatattgtagtagatgttacaattttgtcgccaaactaaacttgctgcttaatgatttgctcacatctagtaaaacatggagtatttgtaaggtgcttggtctcctctataactacaagtatacattggaagcataaagatcaaaccgttggttgcataggatgtcacctttatttaacccattaatactctggttgacctaatcttattctcagacctcaagtgtctgtgcagtatctgttccatttaaatatcagctttacaattatgtggtagcctacacacataatctcatttcatcgctgtaaccaccctgttgtgataaccactattattttacccatcgtacagctgaggaagcaaacagattaagtaacttgcccaaaccagtaaatagcagacctcagactgccacccactgtccttttataatacaatttacagctatattttactttaagcaattcttttattcaaaaaccatttattaagtgcccttgcaatatcaatcgctgtgccaggcattgaatctacagatgtgagcaagacaaagtacctgtcctcaaggagctcatagtataatgaggagattaacaagaaaatgtattattacaatttagtccagtgtcatagcataaggatgatgcgaggggaaaacccgagcagtgttgccaagaggaggaaataggccaatgtggtctgggacggttggatatacttaaacatcttaataatcagagtaattttcatttacaaagagaggtcggtacttaaaataaccctgaaaaataacactggaattccttttctagcattatatttattcctgatttgcctttgccatataatctaatgcttgtttatatagtgtctggtattgtttaacagttctgtcttttctatttaaatgccactaaattttaaattcatacctttccatgattcaaaattcaaaagatcccatgggagatggttggaaaatctccacttcatcctccaagccattcaagtttcctttccagaagcaactgctactgcctttcattcatatgttcttctaaagatagtctacatttggaaatgtatgttaaaagcacgtatttttaaaatttttttcctaaatagtaacacattgtatgtctgctgtgtactttgctatttttatttattttagtgtttcttatatagcagatggaatgaatttgaagttcccagggctgaggatccatgccttctttgtttctaagttatctttcccatagcttttcattatctttcatatgatccagtatatgttaaatatgtcctacatatacatttagacaaccaccatttgttaagtatttgctctaggacagagtttggatttgtttatgtttgctcaaaaggagacccatgggctctccagggtgcactgagtcaatctagtcctaaaaagcaatcttattattaactctgtatgacagaatcatgtctggaacttttgttttctgctttctgtcaagtataaacttcactttgatgctgtacttgcaaaatcacattttctttctggaaattccggcagtgtaccttgactgctagctaccctgtgccagaaaagcctcattcgttgtgcttgaacccttgaatgccaccagctgtcatcactacacagccctcctaagaggcttcctggaggtttcgagattcagatgccctgggagatcccagagtttcctttccctcttggccatattctggtgtcaatgacaaggagtaccttggctttgccacatgtcaaggctgaagaaacagtgtctccaacagagctccttgtgttatctgtttgtacatgtgcatttgtacagtaattggtgtgacagtgttctttgtgtgaattacaggcaagaattgtggctgagcaaggcacatagtctactcagtctattcctaagtcctaactcctccttgtggtgttggatttgtaaggcactttatcccttttgtctcatgtttcatcgtaaatggcataggcagagatgatacctaattctgcatttgattgtcactttttgtacctgcattaatttaataaaatattcttatttattttgttacttggtacaccagcatgtccattttcttgtttattttgtgtttaataaaatgttcagtttaacatcccagtggagaaagttaaaaaa

SEQ ID NO: 29 - protein, 290 aa, human
MRIFAVFIFMTYWHLLNAFTVTVPKDLYVVEYGSNMTIECKFPVEKQLDLAALIVYWEMEDKNIIQFVHGEEDLKVQHSSYRQRARLLKDQLSLGNAALQITDVKLQDAGVYRCMISYGGADYKRITVKVNAPYNKINQRILVVDPVTSEHELTCQAEGYPKAEVIWTSSDHQVLSGKTTTTNSKREEKLFNVTSTLRINTTTNEIFYCTFRRLDPEENHTAELVIPELPLAHPPNERTHLVILGAILLCLGVALTFIFRLRKGRMMDVKKCGIQDTNSKKQSDTHLEET

SEQ ID NO: 30 - DNA, 344 bp, Artificial Sequence
gcgtttactgtcacggttcccaaggacctatatgtggtagagtatggtagcaatatgacaattgaatgcaaattcccagtagaaaaacaattagatctggctgcactaattgtctattgggaaatggaggataagaacattattcaatttgtgcatggagaggaagacctgaaggttcagcatagtagctacagacagagggcccggctgttgaaggaccagctctccctgggaaatgctgcacttcagatcacagatgtgaaattgcaggatgcaggggtgtaccgctgcatgatcagctatggtggtgccgactacaagcgaattactgtgaaagtcaatgg

SEQ ID NO: 31 - DNA, 873 bp, Artificial Sequence
atgaggatatttgctggcattatattcacagcctgctgtcacttgctacgggcgtttactgtcacggttcccaaggacctatatgtggtagagtatggtagcaatatgacaattgaatgcaaattcccagtagaaaaacaattagatctggctgcactaattgtctattgggaaatggaggataagaacattattcaatttgtgcatggagaggaagacctgaaggttcagcatagtagctacagacagagggcccggctgttgaaggaccagctctccctgggaaatgctgcacttcagatcacagatgtgaaattgcaggatgcaggggtgtaccgctgcatgatcagctatggtggtgccgactacaagcgaattactgtgaaagtcaatgccccataccgcaaaatcaaccagagaatttccgtggatccagccacttctgagcatgaactaatatgtcaggccgagggttatccagaagctgaggtaatctggacaaacagtgaccaccaacccgtgagtgggaagagaagtgtcaccacttcccggacagaggggatgcttctcaatgtgaccagcagtctgagggtcaacgccacagcgaatgatgttttctactgtacgttttggagatcacagccagggcaaaaccacacagcggagctgatcatcccagaactgcctgcaacacatcctccacagaacaggactcactgggtgcttctgggatccatcctgttgttcctcattgtagtgtccacggtcctcctcttcttgagaaaacaagtgagaatgctagatgtggagaaatgtggcgttgaagatacaagctcaaaaaaccgaaatgatacacaattcgaggagacgtaa

SEQ ID NO: 32 - DNA, 3653 bp, Artificial Sequence
gaaatcgtggtccccaagcctcatgccaggctgcacttgcacgtcgcgggccagtctcctcgcctgcagatagttcccaaaacatgaggatatttgctggcattatattcacagcctgctgtcacttgctacgggcgtttactgtcacggttcccaaggacctatatgtggtagagtatggtagcaatatgacaattgaatgcaaattcccagtagaaaaacaattagatctggctgcactaattgtctattgggaaatggaggataagaacattattcaatttgtgcatggagaggaagacctgaaggttcagcatagtagctacagacagagggcccggctgttgaaggaccagctctccctgggaaatgctgcacttcagatcacagatgtgaaattgcaggatgcaggggtgtaccgctgcatgatcagctatggtggtgccgactacaagcgaattactgtgaaagtcaatgccccataccgcaaaatcaaccagagaatttccgtggatccagccacttctgagcatgaactaatatgtcaggccgagggttatccagaagctgaggtaatctggacaaacagtgaccaccaacccgtgagtgggaagagaagtgtcaccacttcccggacagaggggatgcttctcaatgtgaccagcagtctgagggtcaacgccacagcgaatgatgttttctactgtacgttttggagatcacagccagggcaaaaccacacagcggagctgatcatcccagaactgcctgcaacacatcctccacagaacaggactcactgggtgcttctgggatccatcctgttgttcctcattgtagtgtccacggtcctcctcttcttgagaaaacaagtgagaatgctagatgtggagaaatgtggcgttgaagatacaagctcaaaaaaccgaaatgatacacaattcgaggagacgtaagcagtgttgaaccctctgatcgtcgattggcagcttgtggtctgtgaaagaaagggcccatgggacatgagtccaaagactcaagatggaacctgagggagagaaccaagaaagtgttgggagaggagcctggaacaacggacattttttccagggagacactgctaagcaagttgcccatcagtcgtcttgggaaatggattgagggttcctggcttagcagctggtccttgcacagtgaccttttcctctgctcagtgccgggatgagagatggagtcatgagtgttgaagaataagtgccttctatttattttgagtctgtgtgttctcactttgggcatgtaattatgactggtgaattctgacgacatgatagatcttaagatgtagtcaccaaactcaactgctgcttagcatcctccgtaactactgatacaagcagggaacacagaggtcacctgcttggtttgacaggctcttgctgtctgactcaaataatctttatttttcagtcctcaaggctcttcgatagcagttgttctgtatcagccttataggtgtcaggtatagcactcaacatctcatctcattacaatagcaaccctcatcaccatagcaacagctaacctctgttatcctcacttcatagccaggaagctgagcgactaagtcacttgcccacagagtatcagctctcagatttctgttcttcagccactgtcctttcaggatagaatttgtcgttaagaaattaatttaaaaactgattattgagtagcattgtatatcaatcacaacatgccttgtgcactgtgctggcctctgagcataaagatgtacgccggagtaccggtcggacatgtttatgtgtgttaaatactcagagaaatgttcattaacaaggagcttgcattttagagacactggaaagtaactccagttcattgtctagcattacatttacctcatttgctatccttgccatacagtctcttgttctccatgaagtgtcatgaatcttgttgaatagttcttttattttttaaatgtttctatttaaatgatattgacatctgaggcgatagctcagttggtaaaaccctttcctcacaagtgtgaaaccctgagtcttatccctagaacccacataaaaaacagttgcgtatgtttgtgcatgcttttgatcccagcactagggaggcagaggcaggcagatcctgagctctcattgaccacccagcctagcctacatggttagctccaggcctacaggagctggcagagcctgaaaaacgatgcctagacacacacacacacacacacacacacacacacacacacacacaccatgtactcatagacctaagtgcaccctcctacacatgcacacacatacaattcaaacacaaatcaacagggaattgtctcagaatggtccccaagacaaagaagaagaaaaacaccaaaccagctctattccctcagcctatcctctctactccttcctagaagcaactactattgtttttgtatataaatttacccaacgacagttaatatgtagaatatatattaaagtgtctgtcaatatatattatctctttctttctttcttcctttctttctttctttctttctttctttctttctttctttctttctttcttccttccttccttccttccttccttccttccttcctttctttctttctttctttttttctgtctatctgtacctaaatggttgctcactatgcattttctgtgctcttcgccctttttatttaatgtatggatatttatgctgcttccagaatggatctaaagctctttgtttctaggttttctcccccatccttctaggcatctctcacactgtctaggccagacaccatgtctgctgcctgaatctgtagacaccatttataaagcacgtactcaccgagtttgtatttggcttgttctgtgtctgattaaagggagaccatgagtccccagggtacactgagttaccccagtaccaagggggagccttgtttgtgtctccatggcagaagcaggcctggagccattttggtttcttccttgacttctctcaaacacagacgcctcacttgctcattacaggttctcctttgggaatgtcagcattgctccttgactgctggctgccctggaaggagcccattagctctgtgtgagcccttgacagctactgcctctccttaccacaggggcctctaagatactgttacctagaggtcttgaggatctgtgttctctggggggaggaaaggaggaggaacccagaactttcttacagttttccttgttctgtcacatgtcaagactgaaggaacaggctgggctacgtagtgagatcctgtctcaaaggaaagacgagcatagccgaacccccggtggaaccccctctgttacctgttcacacaagcttattgatgagtctcatgttaatgtcttgtttgtatgaagtttaagaaaatatcgggttgggcaacacattctatttattcattttatttgaaatcttaatgccatctcatggtgttggattggtgtggcactttattcttttgtgttgtgtataaccataaattttattttgcatcagattgtcaatgtattgcattaatttaataaatatttttatttattaaaaaaaaaaaaaaaaa

SEQ ID NO: 33 - protein, 290 aa, Artificial Sequence
MRIFAGIIFTACCHLLRAFTVTVPKDLYVVEYGSNMTIECKFPVEKQLDLAALIVYWEMEDKNIIQFVHGEEDLKVQHSSYRQRARLLKDQLSLGNAALQITDVKLQDAGVYRCMISYGGADYKRITVKVNAPYRKINQRISVDPATSEHELICQAEGYPEAEVIWTNSDHQPVSGKRSVTTSRTEGMLLNVTSSLRVNATANDVFYCTFWRSQPGQNHTAELIIPELPATHPPQNRTHWVLLGSILLFLIVVSTVLLFLRKQVRMLDVEKCGVEDTSSKNRNDTQFEET

SEQ ID NO: 34 - DNA, 1625 bp, Artificial Sequence
atcatgtggaataggtgcgaggcagaggtgagattttaatggggaggaagcattgaaaagtgaaagtgaaaattggatgctctttgctttgaagctttgcctaaagcaggttttagctttcaaatacgtttcaatgttgaaagaacgcatgatacatatggaggggggcctggggggggtccttggctgagtttgaatgtacattaacaatctggggggctaataactcaatgtaaagctgctgatcccatcatactgacttctttccacttggttctacatggctttgagttacaaaatgaaagcattgaattttgaactgttcagctgtgtttccacacttgcaaatcggttgttggccagccctcagaattgcttcagttacagctggctcgtctgctctttccagactggcttttagggcttatgtatatatgagaaggacacatttactagtgtctccttgctctgctattgaaattaagcagacctctctgtgtttcccgttactagatagttcccaaaacatgaggatatttgctggcattatattcacagcctgctgtcacttgctacggggtaagtcaccaaatcttttcagtgggttctatattttcaatattttagctatgaattaaaaatggaagtaatttgtggggtgtgtatgtgtgtgtatatgtgtgtgtagaggggggtctgtgtgtatgtgcagttgctaggcacacataaagcgttcataggacaacctagagcttagtcctcaccttctaccttgtttgagacaaggtctcttatttgttgtacattgctgagtcctgtagttcggctagctcagaacctcctgggggctctcctgtctccacctcccagtccactgagattgtaggcacatgctactgcacctggcttctacctggtctctggggatttgaacttgggtccatgggctacacagcaagtcgtttacttactgggcaatcactccatcccctaagataattataaggaatataccttgcttatccaaacacattctcattctcctttgccataaataagttacttggcaaatatattgtatgtatttttaataaataaataaaatcttaaaaataaataaaattatttgtgaagacaaaaaaaataagttacttggaaaggatgaaggaaaatactggagctttgggtgtggtttagtagtagaacacttggctgatgtaaaaaaaaagccctaggtgcaatcccaacaccagaaacaaatgaaggaatgaacaacaaccgcccccaccccccaggggatgaatataaaaatatcaggtaatacagaactaacaggtgatccgtttcctatgaataactactgaacattcccagggaggtggcccactgataatatatttttatttattggttccttttaaacaagactgggaatatattatctagcttgcatcaccaccaccaccccccacccccgccccatgaagttatttcaaagaagaattttagtgttcatgtgattccctaaataaaatgatagtaaccttttacccaggttttcagatgtgtttggaggagttttctgtcttctgagggctggtcctctttccttttcagcgtttact

SEQ ID NO: 35 - DNA, 53 bp, Artificial Sequence
gaatacctttaagaaggagatatacatgatcatgtggaataggtgcgaggcag

SEQ ID NO: 36 - DNA, 39 bp, Artificial Sequence
gaaccgtgacagtaaacgctgaaaaggaaagaggaccag

SEQ ID NO: 37 - DNA, 324 bp, Artificial Sequence
gtcacggttcccaaggacctatatgtggtagagtatggtagcaatatgacaattgaatgcaaattcccagtagaaaaacaattagatctggctgcactaattgtctattgggaaatggaggataagaacattattcaatttgtgcatggagaggaagacctgaaggttcagcatagtagctacagacagagggcccggctgttgaaggaccagctctccctgggaaatgctgcacttcagatcacagatgtgaaattgcaggatgcaggggtgtaccgctgcatgatcagctatggtggtgccgactacaagcgaattactgtg

SEQ ID NO: 38 - DNA, 51 bp, Artificial Sequence
ctctttccttttcagcgtttactgtcacggttcccaaggacctatatgtgg

SEQ ID NO: 39 - DNA, 54 bp, Artificial Sequence
cccaatagacaattagtgcagccagatctaattgtttttctactgggaatttgc

SEQ ID NO: 40 - DNA, 35 bp, Artificial Sequence
caattagatctggctgcactaattgtctattggga

SEQ ID NO: 41 - DNA, 43 bp, Artificial Sequence
cttaccattgactttcacagtaattcgcttgtagtcggcacca

SEQ ID NO: 42 - DNA, 1153 bp, Artificial Sequence
aaagtcaatggtaagaattaccctggatggggaaggcttcatccgtatttaaaacagctccctaatgttgagagctcttcattcttgagagttcgcacgcacttctcacagaacaacagcagcctgttcttctcgctcgtttgttcattcgttcgttcacacacttcaccagtgaaaaagcctagcactgtgtgtttgatagtaacttgagattcagtaccagataatactcagccatgctttgcagtcagtaccatgatcttgcaaaggtgaaatgccaggtgtttgtttcttatcataaatgcaatatataatatattacatagatgtatagatataactgtgtaacatgcaataagatataatatgcatatatttcatataacataatgtataatatataatgtataataatatatactacaatatatagttatatgcatagttatatattgcatttatgataaaaagcaaacacctggcatttcacttttgcaagctttttgaattacttgtaaatatatatacatgcaaacatacatacacacacatgtttttttacaagtaatttgaatgtcatggaaagaaatagaatcataaaaatgtccctcctccctaactaccatcttctaagcataaatatacagtaactactatttgtacatccctccatgactttttgattggattactgtttatatttaatctatcaggcttagcacattttctttcctttgaatacctccatacaaaattcaatgtgtgtttatatatatatgtatatatatagttatatcatatcatatatcatacaaagttttatatatgtatacatatataaacacacatatctacacatacatacacattttttatatatatacacaatatataatgtatatgtgtgtgtgtgtgcatatacctctatatctatctatctatctatctatctatctatctatctatctatctatctatagcttctactgtaagggtcactttttaaaaaattaaggttaatctatgaaggatgagaagtgaagatcttaagtgtagaagaagccgttcttccacagagatggtacaggctacactcagcaggcatgcattcattttcagggcctgcatctctgggagtgctgaggaggaacta

SEQ ID NO: 43 - DNA, 45 bp, Artificial Sequence
gcgaattactgtgaaagtcaatggtaagaattaccctggatgggg

SEQ ID NO: 44 - DNA, 53 bp, Artificial Sequence
gcgtcggttgttagcagccggatctcagtagttcctcctcagcactcccagag

SEQ ID NO: 45 - DNA, 25 bp, Artificial Sequence
tggaagaatggctcctgtttcccac

SEQ ID NO: 46 - DNA, 25 bp, Artificial Sequence
cacccctgcatcctgcaatttcaca

SEQ ID NO: 47 - DNA, 25 bp, Artificial Sequence
attagatctggctgcactaattgtc

SEQ ID NO: 48 - DNA, 25 bp, Artificial Sequence
atgagtgaagctctcaggtctatgc

SEQ ID NO: 49 - DNA, 25 bp, Artificial Sequence
atcatgtggaataggtgcgaggcag

SEQ ID NO: 50 - DNA, 25 bp, Artificial Sequence
gaaagagcagacgagccagctgtaa

SEQ ID NO: 51 - DNA, 25 bp, Artificial Sequence
cagactaacactcactccctgctgc

SEQ ID NO: 52 - DNA, 25 bp, Artificial Sequence
aaacatcattcgctgtggcgttgac

SEQ ID NO: 53 - DNA, 20 bp, Artificial Sequence
ctggacctgcttgcgttagt

SEQ ID NO: 54 - DNA, 20 bp, Artificial Sequence
cgtctgtgatctgaagggca

SEQ ID NO: 55 - DNA, 20 bp, Artificial Sequence
ttagatctggctgcactaat

SEQ ID NO: 56 - DNA, 20 bp, Artificial Sequence
agtgcagcatttcccaggga

SEQ ID NO: 57 - DNA, 45 bp, Artificial Sequence
gcatcaagcttggtaccgataggtgcaatcccaacaccagaaaca

SEQ ID NO: 58 - DNA, 45 bp, Artificial Sequence
acttaatcgtggaggatgatagtgcgtgcgaactctcaagaatga

SEQ ID NO: 59 - DNA, 25 bp, Artificial Sequence
ccagggaggtggcccactgataata

SEQ ID NO: 60 - DNA, 25 bp, Artificial Sequence
actaacgcaagcaggtccagctccc

SEQ ID NO: 61 - DNA, 25 bp, Artificial Sequence
cttccacatgagcgtggtcagggcc

SEQ ID NO: 62 - DNA, 25 bp, Artificial Sequence
ccaagggactattttagatgggcag

SEQ ID NO: 63 - DNA, 26 bp, Artificial Sequence
gaagctacaagctcctaggtaggggg

SEQ ID NO: 64 - DNA, 23 bp, Artificial Sequence
acgggttggctcaaaccattaca

SEQ ID NO: 65 - DNA, 20 bp, Artificial Sequence
cctggctcacagtgtcagag

SEQ ID NO: 66 - DNA, 20 bp, Artificial Sequence
cagggctctcctcgattttt

SEQ ID NO: 67 - DNA, 20 bp, Artificial Sequence
ccctgctcgtggtgaccgaa

SEQ ID NO: 68 - DNA, 20 bp, Artificial Sequence
gcaggctctctttgatctgc